European Patent Application EP 4 624 487 A1, published October 1, 2025. Title: PRODUCTION OF ANTIBODIES AGAINST PROTEIN. Applicant: TOKUSHIMA UNIVERSITY. Application JP PCT/JP2023/042024, filed November 22, 2023. The sequence listing filed with the application follows.

SEQUENCE LISTING (146 sequences)

SEQ ID NO: 1 - protein, 15 aa, synthetic construct
GLYLIYSQVLFKGQG

SEQ ID NO: 2 - protein, 15 aa, synthetic construct
KGQGCPSTHVLLTHT

SEQ ID NO: 3 - protein, 15 aa, synthetic construct
YEPIYLGGVFQLEKG

SEQ ID NO: 4 - protein, 15 aa, synthetic construct
LGGVFQLEKGDRLSA

SEQ ID NO: 5 - protein, 15 aa, synthetic construct
PDYLDFAESGQVYFG

SEQ ID NO: 6 - protein, 9 aa, synthetic construct
SYQTKVNLL

SEQ ID NO: 7 - protein, 9 aa, synthetic construct
KPWYEPIYL

SEQ ID NO: 8 - protein, 9 aa, synthetic construct
IYLGGVFQL

SEQ ID NO: 9 - protein, 9 aa, synthetic construct
FQLEKGDRL

SEQ ID NO: 10 - protein, 9 aa, synthetic construct
QVYFGIIAL

SEQ ID NO: 11 - protein, 15 aa, synthetic construct
VRSSSRTPSDKPVAH

SEQ ID NO: 12 - protein, 15 aa, synthetic construct
SDKPVAHVVANPQAE

SEQ ID NO: 13 - protein, 15 aa, synthetic construct
VVANPQAEGQLQWLN

SEQ ID NO: 14 - protein, 15 aa, synthetic construct
GQLQWLNRRANALLA

SEQ ID NO: 15 - protein, 15 aa, synthetic construct
RRANALLANGVELRD

SEQ ID NO: 16 - protein, 15 aa, synthetic construct
NGVELRDNQLVVPSE

SEQ ID NO: 17 - protein, 15 aa, synthetic construct
NQLVVPSEGLYLIYS

SEQ ID NO: 18 - protein, 15 aa, synthetic construct
LTHTISRIAVSYQTK

SEQ ID NO: 19 - protein, 15 aa, synthetic construct
VNLLSAIKSPCQRET

SEQ ID NO: 20 - protein, 15 aa, synthetic construct
PCQRETPEGAEAKPW

SEQ ID NO: 21 - protein, 15 aa, synthetic construct
DRLSAEINRPDYLDF

SEQ ID NO: 22 - protein, 15 aa, synthetic construct
DKPVAHVVANPQAEG

SEQ ID NO: 23 - protein, 15 aa, synthetic construct
VAHVVANPQAEGQLQ

SEQ ID NO: 24 - protein, 15 aa, synthetic construct
AHVVANPQAEGQLQW

SEQ ID NO: 25 - protein, 15 aa, synthetic construct
EGQLQWLNRRANALL

SEQ ID NO: 26 - protein, 15 aa, synthetic construct
LQWLNRRANALLANG

SEQ ID NO: 27 - protein, 15 aa, synthetic construct
RANALLANGVELRDN

SEQ ID NO: 28 - protein, 15 aa, synthetic construct
ANGVELRDNQLVVPS

SEQ ID NO: 29 - protein, 15 aa, synthetic construct
QLVVPSEGLYLIYSQ

SEQ ID NO: 30 - protein, 15 aa, synthetic construct
SEGLYLIYSQVLFKG

SEQ ID NO: 31 - protein, 15 aa, synthetic construct
EGLYLIYSQVLFKGQ

SEQ ID NO: 32 - protein, 15 aa, synthetic construct
SQVLFKGQGCPSTHV

SEQ ID NO: 33 - protein, 15 aa, synthetic construct
QVLFKGQGCPSTHVL

SEQ ID NO: 34 - protein, 15 aa, synthetic construct
STHVLLTHTISRIAV

SEQ ID NO: 35 - protein, 15 aa, synthetic construct
HVLLTHTISRIAVSY

SEQ ID NO: 36 - protein, 15 aa, synthetic construct
THTISRIAVSYQTKV

SEQ ID NO: 37 - protein, 15 aa, synthetic construct
ISRIAVSYQTKVNLL

SEQ ID NO: 38 - protein, 15 aa, synthetic construct
RIAVSYQTKVNLLSA

SEQ ID NO: 39 - protein, 15 aa, synthetic construct
QTKVNLLSAIKSPCQ

SEQ ID NO: 40 - protein, 15 aa, synthetic construct
KVNLLSAIKSPCQRE

SEQ ID NO: 41 - protein, 15 aa, synthetic construct
LSAIKSPCQRETPEG

SEQ ID NO: 42 - protein, 15 aa, synthetic construct
PIYLGGVFQLEKGDR

SEQ ID NO: 43 - protein, 15 aa, synthetic construct
LGGVFQLEKGDRLSA

SEQ ID NO: 44 - protein, 15 aa, synthetic construct
VFQLEKGDRLSAEIN

SEQ ID NO: 45 - protein, 15 aa, synthetic construct
GDRLSAEINRPDYLD

SEQ ID NO: 46 - protein, 15 aa, synthetic construct
YLDFAESGQVYFGII

SEQ ID NO: 47 - protein, 14 aa, synthetic construct
DAEFRHDSGYEVHH

SEQ ID NO: 48 - protein, 14 aa, synthetic construct
QKLVFFAEDVGSNK

SEQ ID NO: 49 - protein, 14 aa, synthetic construct
GAIIGLMVGGVVIA

SEQ ID NO: 50 - protein, 14 aa, synthetic construct
SGYEVHHQKLVFFA

SEQ ID NO: 51 - protein, 14 aa, synthetic construct
EDVGSNKGAIIGLM

SEQ ID NO: 52 - protein, 9 aa, synthetic construct
LDFAESGQV

SEQ ID NO: 53 - protein, 15 aa, synthetic construct
DFAESGQVYFGIIAL

SEQ ID NO: 54 - protein, 157 aa, Homo sapiens [sequence omitted]

SEQ ID NO: 55 - protein, 15 aa, Mouse
GWLLEVPNGPWRSLT

SEQ ID NO: 56 - protein, 15 aa, Mouse
ATFTCSLSNWSEDLM

SEQ ID NO: 57 - protein, 15 aa, Mouse
KQAAFCNGLSQPVQD

SEQ ID NO: 58 - protein, 15 aa, Mouse
FHMNILDTRRNDSGI

SEQ ID NO: 59 - RNA, 45 nt, synthetic construct
  source 1..45: mol_type = other RNA
gggcagctccagtggctgaaccgccgggccaatgccctcctggcc

SEQ ID NO: 60 - RNA, 45 nt, synthetic construct
  source 1..45: mol_type = other RNA
ccctgccagagggagaccccagagggggctgaggccaagccctgg

SEQ ID NO: 61 - RNA, 45 nt, synthetic construct
  source 1..45: mol_type = other RNA
ctccagtggctgaaccgccgggccaatgccctcctggccaatggc

SEQ ID NO: 62 - RNA, 45 nt, synthetic construct
  source 1..45: mol_type = other RNA
gactttgccgagtctgggcaggtctactttgggatcattgccctg

SEQ ID NO: 63 - RNA, 42 nt, synthetic construct
  source 1..42: mol_type = other RNA
tcaggatatgaagttcatcatcaaaaattggtgttctttgca

SEQ ID NO: 64 - protein, 157 aa, synthetic construct
VRSSSRTPSDKPVAHVVANPQAEGQLQWLNRRANALLANGVELRDNQLVVPSEGLYLIYSQVLFKGQGCPSTHVLLTHTISRIAVSYQTKANLLSAIKSPCQRETPEGAEAKPWYEPIYLGGVFQLEKGDRLSAEINRPDYLDFAESGQVYFGIIAL

SEQ ID NO: 65 - DNA, 471 bp, synthetic construct
  source 1..471: mol_type = other DNA
gtcagatcatcttctcgaaccccgagtgacaagcctgtagcccatgttgtagcaaaccctcaagctgaggggcagctccagtggctgaaccgccgggccaatgccctcctggccaatggcgtggagctgagagataaccagctggtggtgccatcagagggcctgtacctcatctactcccaggtcctcttcaagggccaaggctgcccctccacccatgtgctcctcacccacaccatcagccgcatcgccgtctcctaccagaccaaggacaacctcctctctgccatcaagagcccctgccagagggagaccccagagggggctgaggccaagccctggtatgagcccatctatctgggaggggtcttccagctggagaagggtgaccgactcagcgctgagatcaatcggcccgactatctcgactttgccgagtctgggcaggtctactttgggatcattgccctg

SEQ ID NO: 66 - protein, 157 aa, synthetic construct
VRSSSRTPSDKPVAHVVANPQAEGQLQWLNRRANALLANGVELRDNQLVVPSEGLYLIYSQVLFKGQGAPSTHVLLTHTISRIAVSYQTKVNLLSAIKSPAQRETPEGAEAKPWYEPIYLGGVFQLEKGDRLSAEINRPDYLDFAESGQVYFGIIAL

SEQ ID NO: 67 - DNA, 471 bp, synthetic construct
  source 1..471: mol_type = other DNA
gtcagatcatcttctcgaaccccgagtgacaagcctgtagcccatgttgtagcaaaccctcaagctgaggggcagctccagtggctgaaccgccgggccaatgccctcctggccaatggcgtggagctgagagataaccagctggtggtgccatcagagggcctgtacctcatctactcccaggtcctcttcaagggccaaggcgccccctccacccatgtgctcctcacccacaccatcagccgcatcgccgtctcctaccagaccaaggtcaacctcctctctgccatcaagagccccgcccagagggagaccccagagggggctgaggccaagccctggtatgagcccatctatctgggaggggtcttccagctggagaagggtgaccgactcagcgctgagatcaatcggcccgactatctcgactttgccgagtctgggcaggtctactttgggatcattgccctg

SEQ ID NO: 68 - protein, 15 aa, Homo sapiens
FLDSPDRPWNPPTFS

SEQ ID NO: 69 - protein, 15 aa, Homo sapiens
CSFSNTSESFVLNWY

SEQ ID NO: 70 - protein, 15 aa, Homo sapiens
EDRSQPGQDCRFRVT

SEQ ID NO: 71 - protein, 15 aa, Homo sapiens
RRNDSGTYLCGAISL

SEQ ID NO: 72 - protein, 15 aa, Homo sapiens
VTERRAEVPTAHPSP

SEQ ID NO: 73 - protein, 15 aa, Homo sapiens
PALLVVTEGDNATFT

SEQ ID NO: 74 - protein, 15 aa, Homo sapiens
RMSPSNQTDKLAAFP

SEQ ID NO: 75 - protein, 15 aa, Homo sapiens
QLPNGRDFHMSVVRA

SEQ ID NO: 76 - protein, 15 aa, Homo sapiens
APKAQIKESLRAELR

SEQ ID NO: 77 - skipped

SEQ ID NO: 78 - protein, 15 aa, Homo sapiens
PSPSPRPAGQFQTLV

SEQ ID NO: 79 - protein, 15 aa, Homo sapiens
PWNPPTFSPALLVVT

SEQ ID NO: 80 - protein, 15 aa, Homo sapiens
ESFVLNWYRMSPSNQ

SEQ ID NO: 81 - protein, 15 aa, Homo sapiens
QDCRFRVTQLPNGRD

SEQ ID NO: 82 - protein, 15 aa, Homo sapiens
YLCGAISLAPKAQIK

SEQ ID NO: 83 - protein, 15 aa, Homo sapiens
VPTAHPSPSPRPAGQ

SEQ ID NO: 84 - protein, 15 aa, Homo sapiens
EGDNATFTCSFSNTS

SEQ ID NO: 85 - protein, 15 aa, Homo sapiens
TDKLAAFPEDRSQPG

SEQ ID NO: 86 - protein, 15 aa, Homo sapiens
FHMSVVRARRNDSGT

SEQ ID NO: 87 - protein, 15 aa, Homo sapiens
ESLRAELRVTERRAE

SEQ ID NO: 88 - protein, 15 aa, Homo sapiens
FTVTVPKDLYVVEYG

SEQ ID NO: 89 - protein, 15 aa, Homo sapiens
DLAALIVYWEMEDKN

SEQ ID NO: 90 - protein, 15 aa, Homo sapiens
SSYRQRARLLKDQLS

SEQ ID NO: 91 - protein, 15 aa, Homo sapiens
AGVYRCMISYGGADY

SEQ ID NO: 92 - protein, 15 aa, Homo sapiens
QRILVVDPVTSEHEL

SEQ ID NO: 93 - protein, 15 aa, Homo sapiens
SSDHQVLSGKTTTTN

SEQ ID NO: 94 - protein, 15 aa, Homo sapiens
INTTTNEIFYCTFRR

SEQ ID NO: 95 - protein, 15 aa, Homo sapiens
LVIPELPLAHPPNER

SEQ ID NO: 96 - protein, 15 aa, Homo sapiens
SNMTIECKFPVEKQL

SEQ ID NO: 97 - protein, 15 aa, Homo sapiens
IIQFVHGEEDLKVQH

SEQ ID NO: 98 - protein, 15 aa, Homo sapiens
LGNAALQITDVKLQD

SEQ ID NO: 99 - protein, 15 aa, Homo sapiens
KRITVKVNAPYNKIN

SEQ ID NO: 100 - protein, 15 aa, Homo sapiens
TCQAEGYPKAEVIWT

SEQ ID NO: 101 - protein, 15 aa, Homo sapiens
SKREEKLFNVTSTLR

SEQ ID NO: 102 - protein, 15 aa, Homo sapiens
LDPEENHTAELVIPE

SEQ ID NO: 103 - protein, 15 aa, Homo sapiens
DLYVVEYGSNMTIEC

SEQ ID NO: 104 - protein, 15 aa, Homo sapiens
YWEMEDKNIIQFVHG

SEQ ID NO: 105 - protein, 15 aa, Homo sapiens
RLLKDQLSLGNAALQ

SEQ ID NO: 106 - protein, 15 aa, Homo sapiens
ISYGGADYKRITVKV

SEQ ID NO: 107 - protein, 15 aa, Homo sapiens
PVTSEHELTCQAEGY

SEQ ID NO: 108 - protein, 15 aa, Homo sapiens
SGKTTTTNSKREEKL

SEQ ID NO: 109 - protein, 15 aa, Homo sapiens
IFYCTFRRLDPEENH

SEQ ID NO: 110 - protein, 15 aa, Homo sapiens
KFPVEKQLDLAALIV

SEQ ID NO: 111 - protein, 15 aa, Homo sapiens
EEDLKVQHSSYRQRA

SEQ ID NO: 112 - protein, 15 aa, Homo sapiens
ITDVKLQDAGVYRCM

SEQ ID NO: 113 - protein, 15 aa, Homo sapiens
NAPYNKINQRILVVD

SEQ ID NO: 114 - protein, 15 aa, Homo sapiens
PKAEVIWTSSDHQVL

SEQ ID NO: 115 - protein, 15 aa, Homo sapiens
FNVTSTLRINTTTNE

SEQ ID NO: 116 - protein, 15 aa, Homo sapiens
TAELVIPELPLAHPP

SEQ ID NO: 117 - protein, 20 aa, Homo sapiens
RPDYLDFAESGQVYFGIIAL

SEQ ID NO: 118 - protein, 25 aa, Homo sapiens
SAEINRPDYLDFAESGQVYFGIIAL

SEQ ID NO: 119 - protein, 30 aa, Homo sapiens
KGDRLSAEINRPDYLDFAESGQVYFGIIAL

SEQ ID NO: 120 - protein, 30 aa, Homo sapiens
VRSSSRTPSDKPVAHVVANPQAEGQLQWLN

SEQ ID NO: 121 - protein, 30 aa, Homo sapiens
PSDKPVAHVVANPQAEGQLQWLNRRANALL

SEQ ID NO: 122 - protein, 30 aa, Homo sapiens
RRANALLANGVELRDNQLVVPSEGLYLIYS

SEQ ID NO: 123 - protein, 30 aa, Homo sapiens
ANGVELRDNQLVVPSEGLYLIYSQVLFKGQ

SEQ ID NO: 124 - protein, 30 aa, Homo sapiens
VNLLSAIKSPCQRETPEGAEAKPWYEPIYL

SEQ ID NO: 125 - protein, 30 aa, Homo sapiens
GGVFQLEKGDRLSAEINRPDYLDFAESGQV

SEQ ID NO: 126 - protein, 30 aa, Homo sapiens; identical to SEQ ID NO: 119

SEQ ID NO: 127 - protein, 157 aa, Homo sapiens
VRSSSRTPSDKPVAHVVANPQAEGQLQWLNRRANALLANGVELRDNQLVVPSEGLYLIYSQVLFKGQGCPSTHVLLTHTISRIAVSYQTKDNLLSAIKSPCQRETPEGAEAKPWYEPIYLGGVFQLEKGDRLSAEINRPDYLDFAESGQVYFGIIAL

SEQ ID NO: 128 - protein, 15 aa, Mouse
MWVRQVPWSFTWAVL

SEQ ID NO: 129 - protein, 15 aa, Mouse
NGPWRSLTFYPAWLT

SEQ ID NO: 130 - protein, 15 aa, Mouse
SNWSEDLMLNWNRLS

SEQ ID NO: 131 - protein, 15 aa, Mouse
GLSQPVQDARFQIIQ

SEQ ID NO: 132 - protein, 15 aa, Mouse
TRRNDSGIYLCGAIS

SEQ ID NO: 133 - protein, 15 aa, Mouse
ELVVTERILETSTRY

SEQ ID NO: 134 - protein, 15 aa, Mouse
LQLSWQSGWLLEVPN

SEQ ID NO: 135 - protein, 15 aa, Mouse
TVSEGANATFTCSLS

SEQ ID NO: 136 - protein, 15 aa, Mouse
SPSNQTEKQAAFCNG

SEQ ID NO: 137 - protein, 15 aa, Mouse
QLPNRHDFHMNILDT

SEQ ID NO: 138 - protein, 15 aa, Mouse
SLHPKAKIEESPGAE

SEQ ID NO: 139 - protein, 15 aa, Mouse
YPSPSPKPEGRFQGM

SEQ ID NO: 140 - protein, 15 aa, Mouse
WSFTWAVLQLSWQSG

SEQ ID NO: 141 - protein, 15 aa, Mouse
TFYPAWLTVSEGANA

SEQ ID NO: 142 - protein, 15 aa, Mouse
MLNWNRLSPSNQTEK

SEQ ID NO: 143 - protein, 15 aa, Mouse
DARFQIIQLPNRHDF

SEQ ID NO: 144 - protein, 15 aa, Mouse
IYLCGAISLHPKAKI

SEQ ID NO: 145 - protein, 15 aa, Mouse
ILETSTRYPSPSPKP

SEQ ID NO: 146 - protein, 15 aa, Mouse
IEESPGAELVVTERI